European Patent Application EP 4 417 623 A1, published August 21, 2024. Title: CCR9 TARGETING MOIETY FOR THE TREATMENT OF CCR9-POSITIVE CANCER. Applicant: FUNDACION INSTITUT DE RECERCA CONTRA LA LEUCEMIA JOSEP CARRERAS. The sequence listing filed with the application follows.

SEQUENCE LISTING (36 sequences)

SEQ ID NO: 1 - protein, 9 aa, synthetic construct
SMEDYVNFN

SEQ ID NO: 2 - protein, 11 aa, synthetic construct
QSLVHSNGKTY

SEQ ID NO: 3 - skipped

SEQ ID NO: 4 - protein, 8 aa, synthetic construct
AQSTHVWT

SEQ ID NO: 5 - protein, 8 aa, synthetic construct
GYSFTDYI

SEQ ID NO: 6 - protein, 8 aa, synthetic construct
IDPNNYNT

SEQ ID NO: 7 - protein, 5 aa, synthetic construct
ARDVY

SEQ ID NO: 8 - protein, 113 aa, synthetic construct
DVVMTQTPLSLSVTPGQPASISCRSSQSLVHSNGKTYLQWYLQKPGQSPKLLIYKVSNRFSGVPDRFSGSGSGTDFTLKISRVEAEDVGVYFCAQSTHVWTFGGGTKVEIKRA

SEQ ID NO: 9 - protein, 112 aa, synthetic construct
QVQLKQSGPEVVKPGTSVKVSCTASGYSFTDYIIYWVKQAHGRSLEWMGYIDPNNYNTRYSQKFQGKVTITVDKSSTSAYMELNSLTSDDTAVYYCARDVYWGQGTTVTVSS

SEQ ID NO: 10 - protein, 113 aa, synthetic construct; identical to SEQ ID NO: 8

SEQ ID NO: 11 - protein, 112 aa, synthetic construct
QVQLVQSGAEVKKPGASVKVSCTASGYSFTDYIIYWVKQAHGQSLEWMGYIDPNNYNTRYSQKFQGKVTITVDKSSTSAYMELNSLTSDDTAVYYCARDVYWGQGTTVTVSS

SEQ ID NO: 12 - protein, 113 aa, synthetic construct
DVVMTQTPLSLTVSLGDQASISCRSSQSLVHSNGKTYLQWYLQKPGQSPKLLIYKVSNRFSGVPDRFSGSGSGTDFTLKISRVEAEDLGVYFCAQSTHVWTFGGGTKLEIKRA

SEQ ID NO: 13 - protein, 112 aa, synthetic construct
QVQLKQSGPELVKPGTSVRVSCTASGYSFTDYIIYWVKQSHGRSLEWIGYIDPNNYNTRYSQKFKGKATLTVDKSSTSAFMHLNSLTSDDSAVYYCARDVYWGQGTTLTVSS

SEQ ID NO: 14 - protein, 20 aa, synthetic construct
GGGGSGGGGSGGGGSGGGGS

SEQ ID NO: 15 - protein, 23 aa, synthetic construct
MALPVTGLLLSLGLLLHAARPTG

SEQ ID NO: 16 - protein, 245 aa, synthetic construct
QVQLKQSGPEVVKPGTSVKVSCTASGYSFTDYIIYWVKQAHGRSLEWMGYIDPNNYNTRYSQKFQGKVTITVDKSSTSAYMELNSLTSDDTAVYYCARDVYWGQGTTVTVSSGGGGSGGGGSGGGGSGGGGSDVVMTQTPLSLSVTPGQPASISCRSSQSLVHSNGKTYLQWYLQKPGQSPKLLIYKVSNRFSGVPDRFSGSGSGTDFTLKISRVEAEDVGVYFCAQSTHVWTFGGGTKVEIKRA

SEQ ID NO: 17 - protein, 245 aa, synthetic construct
QVQLVQSGAEVKKPGASVKVSCTASGYSFTDYIIYWVKQAHGQSLEWMGYIDPNNYNTRYSQKFQGKVTITVDKSSTSAYMELNSLTSDDTAVYYCARDVYWGQGTTVTVSSGGGGSGGGGSGGGGSGGGGSDVVMTQTPLSLSVTPGQPASISCRSSQSLVHSNGKTYLQWYLQKPGQSPKLLIYKVSNRFSGVPDRFSGSGSGTDFTLKISRVEAEDVGVYFCAQSTHVWTFGGGTKVEIKRA

SEQ ID NO: 18 - protein, 245 aa, synthetic construct
QVQLKQSGPELVKPGTSVRVSCTASGYSFTDYIIYWVKQSHGRSLEWIGYIDPNNYNTRYSQKFKGKATLTVDKSSTSAFMHLNSLTSDDSAVYYCARDVYWGQGTTLTVSSGGGGSGGGGSGGGGSGGGGSDVVMTQTPLSLTVSLGDQASISCRSSQSLVHSNGKTYLQWYLQKPGQSPKLLIYKVSNRFSGVPDRFSGSGSGTDFTLKISRVEAEDLGVYFCAQSTHVWTFGGGTKLEIKRA

SEQ ID NO: 19 - protein, 69 aa, synthetic construct
TTTPAPRPPTPAPTIASQPLSLRPEACRPAAGGAVHTRGLDFACDIYIWAPLAGTCGVLLLSLVITLYC

SEQ ID NO: 20 - protein, 113 aa, synthetic construct
RVKFSRSADAPAYQQGQNQLYNELNLGRREEYDVLDKRRGRDPEMGGKPQRRKNPQEGLYNELQKDKMAEAYSEIGMKGERRRGKGHDGLYQGLSTATKDTYDALHMQALPPR

SEQ ID NO: 21 - protein, 42 aa, synthetic construct
KRGRKKLLYIFKQPFMRPVQTTQEEDGCSCRFPEEEEGGCEL

SEQ ID NO: 22 - protein, 492 aa, synthetic construct
MALPVTGLLLSLGLLLHAARPTGQVQLKQSGPELVKPGTSVRVSCTASGYSFTDYIIYWVKQSHGRSLEWIGYIDPNNYNTRYSQKFKGKATLTVDKSSTSAFMHLNSLTSDDSAVYYCARDVYWGQGTTLTVSSGGGGSGGGGSGGGGSGGGGSDVVMTQTPLSLTVSLGDQASISCRSSQSLVHSNGKTYLQWYLQKPGQSPKLLIYKVSNRFSGVPDRFSGSGSGTDFTLKISRVEAEDLGVYFCAQSTHVWTFGGGTKLEIKRATTTPAPRPPTPAPTIASQPLSLRPEACRPAAGGAVHTRGLDFACDIYIWAPLAGTCGVLLLSLVITLYCKRGRKKLLYIFKQPFMRPVQTTQEEDGCSCRFPEEEEGGCELRVKFSRSADAPAYQQGQNQLYNELNLGRREEYDVLDKRRGRDPEMGGKPQRRKNPQEGLYNELQKDKMAEAYSEIGMKGERRRGKGHDGLYQGLSTATKDTYDALHMQALPPR

SEQ ID NO: 23 - protein, 492 aa, synthetic construct
MALPVTGLLLSLGLLLHAARPTGQVQLKQSGPEVVKPGTSVKVSCTASGYSFTDYIIYWVKQAHGRSLEWMGYIDPNNYNTRYSQKFQGKVTITVDKSSTSAYMELNSLTSDDTAVYYCARDVYWGQGTTVTVSSGGGGSGGGGSGGGGSGGGGSDVVMTQTPLSLSVTPGQPASISCRSSQSLVHSNGKTYLQWYLQKPGQSPKLLIYKVSNRFSGVPDRFSGSGSGTDFTLKISRVEAEDVGVYFCAQSTHVWTFGGGTKVEIKRATTTPAPRPPTPAPTIASQPLSLRPEACRPAAGGAVHTRGLDFACDIYIWAPLAGTCGVLLLSLVITLYCKRGRKKLLYIFKQPFMRPVQTTQEEDGCSCRFPEEEEGGCELRVKFSRSADAPAYQQGQNQLYNELNLGRREEYDVLDKRRGRDPEMGGKPQRRKNPQEGLYNELQKDKMAEAYSEIGMKGERRRGKGHDGLYQGLSTATKDTYDALHMQALPPR

SEQ ID NO: 24 - protein, 492 aa, synthetic construct
MALPVTGLLLSLGLLLHAARPTGQVQLVQSGAEVKKPGASVKVSCTASGYSFTDYIIYWVKQAHGQSLEWMGYIDPNNYNTRYSQKFQGKVTITVDKSSTSAYMELNSLTSDDTAVYYCARDVYWGQGTTVTVSSGGGGSGGGGSGGGGSGGGGSDVVMTQTPLSLSVTPGQPASISCRSSQSLVHSNGKTYLQWYLQKPGQSPKLLIYKVSNRFSGVPDRFSGSGSGTDFTLKISRVEAEDVGVYFCAQSTHVWTFGGGTKVEIKRATTTPAPRPPTPAPTIASQPLSLRPEACRPAAGGAVHTRGLDFACDIYIWAPLAGTCGVLLLSLVITLYCKRGRKKLLYIFKQPFMRPVQTTQEEDGCSCRFPEEEEGGCELRVKFSRSADAPAYQQGQNQLYNELNLGRREEYDVLDKRRGRDPEMGGKPQRRKNPQEGLYNELQKDKMAEAYSEIGMKGERRRGKGHDGLYQGLSTATKDTYDALHMQALPPR

SEQ ID NO: 25 - protein, 11 aa, synthetic construct
QASQDINKYIA

SEQ ID NO: 26 - protein, 7 aa, synthetic construct
IHYTSTL

SEQ ID NO: 27 - protein, 9 aa, synthetic construct
LHYDNLPWT

SEQ ID NO: 28 - protein, 11 aa, synthetic construct
SGYAFSTYTMH

SEQ ID NO: 29 - protein, 10 aa, synthetic construct
YINPNSASTS

SEQ ID NO: 30 - protein, 9 aa, synthetic construct
ARGFYTMDY

SEQ ID NO: 31 - protein, 110 aa, synthetic construct
RDIQMTQSPSSLSASVGDRVTITCQASQDINKYIAWYQFKPGKGPRLLIHYTSTLEPAIPSRFSGSGSGREYTFTISSLQPEDIATYYCLHYDNLPWTFGGGTKVEIKRA

SEQ ID NO: 32 - protein, 116 aa, synthetic construct
QVQLQQSGAEVKKPGASVKVSCKASGYAFSTYTMHWVRQAPGQGLEWMGYINPNSASTSYAQKFQGRVTMTADKSTNTAYMELSSLRSEDTAVYYCARGFYTMDYWGQGTLVTVSS

SEQ ID NO: 33 - protein, 109 aa, synthetic construct
DIQMTQSPSSVSASVGDRVTISCQASQDINKYIAWYQFKPGKGPRLLIHYTSTLQPAIPSRFSGSGSGREYTLTISSLQPEDFATYYCLHYDNLPWTFGGGTKVEVRRA

SEQ ID NO: 34 - protein, 117 aa, synthetic construct
QVQLVQSGPEVAKPGASVRLSCKASGYAFSTYTMHWVRQAPGQGLEWMGYINPNSASTSYNQNFKARVTLTADKSTNTAYMHLSSLTSDDTAVYYCGRGFYTMDYWGQGTLVTVSSA

SEQ ID NO: 35 - protein, 246 aa, synthetic construct
QVQLQQSGAEVKKPGASVKVSCKASGYAFSTYTMHWVRQAPGQGLEWMGYINPNSASTSYAQKFQGRVTMTADKSTNTAYMELSSLRSEDTAVYYCARGFYTMDYWGQGTLVTVSSGGGGSGGGGSGGGGSGGGGSRDIQMTQSPSSLSASVGDRVTITCQASQDINKYIAWYQFKPGKGPRLLIHYTSTLEPAIPSRFSGSGSGREYTFTISSLQPEDIATYYCLHYDNLPWTFGGGTKVEIKRA

SEQ ID NO: 36 - protein, 246 aa, synthetic construct
QVQLVQSGPEVAKPGASVRLSCKASGYAFSTYTMHWVRQAPGQGLEWMGYINPNSASTSYNQNFKARVTLTADKSTNTAYMHLSSLTSDDTAVYYCGRGFYTMDYWGQGTLVTVSSAGGGGSGGGGSGGGGSGGGGSDIQMTQSPSSVSASVGDRVTISCQASQDINKYIAWYQFKPGKGPRLLIHYTSTLQPAIPSRFSGSGSGREYTLTISSLQPEDFATYYCLHYDNLPWTFGGGTKVEVRRA